European Patent Application EP 4 279 598 A2, published November 22, 2023. Title: Nepentesin-1 derived resistance to fungal pathogens in major crop plants. Applicant: Aarhus University. The sequence listing filed with the application follows.

SEQUENCE LISTING (55 sequences)

SEQ ID NO: 1 - DNA, 1359 bp, Hordeum vulgare
  source 1..1359: mol_type = genomic DNA
  CDS 1..1359: note = HvNep-1 gene encoding HvNEP1 aspartic protease
atggccatggccatcatgaacaccctccagtgcatcctcttcctcatggccctcatcatgacccaccagatcccgcgcgccaccgccgatgcggacaccccaaaagtcgccatggctagctcgggcgccggttcgagcttccggctggcggcccatcatgaccacgcgctgagccggagcgacgacggcttcctccatgtccagagccggctggacaaccttcttccatcggaggcgaacgtcaccaccctccgcccaccagtggcctcgccgctcgatatggccttcagcgtggtcgttggcttgggctcgggcaaaggccggcatgactacaacctcaagctcgacgcctctggtagcctgacatgggtgcaatgcaagccctgcaatcccaagcagccacagcgcggccccctgttcgatcccaaggcctcgtccaccttccagcaagtggccggcacgagccagatttgccacccgccgtaccccatggagcccgcggggcagcagtgcgccttccacctgtccggcatgggcggcatgtcggtgcatggctacgtggccatggagaacctcaccatggggccagaggcaatgaaggagttcgtcttcgggtgctcgcactcgacggggcacttcaacagccacggcaccttcgcgggcgtcgccgccatgggcaagatgcccacctcgctcgtcatgcaggtggcggcgcgcgggcagacgcggttctcgtactgcctcttctccggcggggcgagccggcatgggttcctccggttcggcgccgacgtgccgagccggtcgggcctccggacgaccaagatcctcccggcgctggacgcgcacgagtcgcagtactacgtgagcctcgtgggcatcagcctggacgccaagaggctgacgggggtcaggccggagatgttcgcccgacagcgcggtggggagggcgggtgcgtggtcgaccccggcacgccgctgacggtgctggtccgggaggcgtaccgcgtcgtggaggacgccgtctggagtgacctacgacggaacaaggccgagcgcgtgcagcgcgaaggctacgggctgtgcgtgcgcaaaaccgcagagatcaagcggcatctgcagtcgctgtccttgcacttcgcggaggagacggcgaggctggtcgtgaagccggagcagctgttcgtggcggtggagagcaggctccatggggccgccctgtgccttgccatgcgtccgggcgagcggacggtcatcggcgcgctgcagcaggtggacacgaggttcgtgtacgacctcaaagacgccaaactgtcctttgcgtccgagccgtgctctcaggacaccgccggtgtggat

SEQ ID NO: 2 - protein, 453 aa, Hordeum vulgare
  source 1..453: note = The sequence is a translation of the CDS of SEQ ID NO. 1
MAMAIMNTLQCILFLMALIMTHQIPRATADADTPKVAMASSGAGSSFRLAAHHDHALSRSDDGFLHVQSRLDNLLPSEANVTTLRPPVASPLDMAFSVVVGLGSGKGRHDYNLKLDASGSLTWVQCKPCNPKQPQRGPLFDPKASSTFQQVAGTSQICHPPYPMEPAGQQCAFHLSGMGGMSVHGYVAMENLTMGPEAMKEFVFGCSHSTGHFNSHGTFAGVAAMGKMPTSLVMQVAARGQTRFSYCLFSGGASRHGFLRFGADVPSRSGLRTTKILPALDAHESQYYVSLVGISLDAKRLTGVRPEMFARQRGGEGGCVVDPGTPLTVLVREAYRVVEDAVWSDLRRNKAERVQREGYGLCVRKTAEIKRHLQSLSLHFAEETARLVVKPEQLFVAVESRLHGAALCLAMRPGERTVIGALQQVDTRFVYDLKDAKLSFASEPCSQDTAGVD

SEQ ID NO: 3 - DNA, 1272 bp, Hordeum vulgare
  source 1..1272: mol_type = genomic DNA
  CDS 1..1272: note = Nucleotide sequence encoding HvNEP (truncated to delete signal peptide)
gatgcggacaccccaaaagtcgccatggctagctcgggcgccggttcgagcttccggctggcggcccatcatgaccacgcgctgagccggagcgacgacggcttcctccatgtccagagccggctggacaaccttcttccatcggaggcgaacgtcaccaccctccgcccaccagtggcctcgccgctcgatatggccttcagcgtggtcgttggcttgggctcgggcaaaggccggcatgactacaacctcaagctcgacgcctctggtagcctgacatgggtgcaatgcaagccctgcaatcccaagcagccacagcgcggccccctgttcgatcccaaggcctcgtccaccttccagcaagtggccggcacgagccagatttgccacccgccgtaccccatggagcccgcggggcagcagtgcgccttccacctgtccggcatgggcggcatgtcggtgcatggctacgtggccatggagaacctcaccatggggccagaggcaatgaaggagttcgtcttcgggtgctcgcactcgacggggcacttcaacagccacggcaccttcgcgggcgtcgccgccatgggcaagatgcccacctcgctcgtcatgcaggtggcggcgcgcgggcagacgcggttctcgtactgcctcttctccggcggggcgagccggcatgggttcctccggttcggcgccgacgtgccgagccggtcgggcctccggacgaccaagatcctcccggcgctggacgcgcacgagtcgcagtactacgtgagcctcgtgggcatcagcctggacgccaagaggctgacgggggtcaggccggagatgttcgcccgacagcgcggtggggagggcgggtgcgtggtcgaccccggcacgccgctgacggtgctggtccgggaggcgtaccgcgtcgtggaggacgccgtctggagtgacctacgacggaacaaggccgagcgcgtgcagcgcgaaggctacgggctgtgcgtgcgcaaaaccgcagagatcaagcggcatctgcagtcgctgtccttgcacttcgcggaggagacggcgaggctggtcgtgaagccggagcagctgttcgtggcggtggagagcaggctccatggggccgccctgtgccttgccatgcgtccgggcgagcggacggtcatcggcgcgctgcagcaggtggacacgaggttcgtgtacgacctcaaagacgccaaactgtcctttgcgtccgagccgtgctctcaggacaccgccggtgtggat

SEQ ID NO: 4 - protein, 424 aa, Hordeum vulgare
  source 1..424: note = The sequence is a translation of the CDS of SEQ ID NO. 3
DADTPKVAMASSGAGSSFRLAAHHDHALSRSDDGFLHVQSRLDNLLPSEANVTTLRPPVASPLDMAFSVVVGLGSGKGRHDYNLKLDASGSLTWVQCKPCNPKQPQRGPLFDPKASSTFQQVAGTSQICHPPYPMEPAGQQCAFHLSGMGGMSVHGYVAMENLTMGPEAMKEFVFGCSHSTGHFNSHGTFAGVAAMGKMPTSLVMQVAARGQTRFSYCLFSGGASRHGFLRFGADVPSRSGLRTTKILPALDAHESQYYVSLVGISLDAKRLTGVRPEMFARQRGGEGGCVVDPGTPLTVLVREAYRVVEDAVWSDLRRNKAERVQREGYGLCVRKTAEIKRHLQSLSLHFAEETARLVVKPEQLFVAVESRLHGAALCLAMRPGERTVIGALQQVDTRFVYDLKDAKLSFASEPCSQDTAGVD

SEQ ID NO: 5 - DNA, 1356 bp, Aegilops tauschii
  source 1..1356: mol_type = genomic DNA
  CDS 1..1356: note = Nep-1 gene encoding NEP-1 aspartic endoprotease
atggccatggcgatcaagagcactctccaatgcgtagtgttcctgatggcgctcatcacgacccacctgataccgcctgccgatgctgatgcgggcagcccaaaagttgccatggctagctcgggcgctggttcaagcttccggctggtagcccaccatgactatgcgctgcgcgacgacggcttcctccacgtccagagccggctggacgaccttcttccatcggaggcgaacgtcaccaccctccgcccaccagtggcctcgccgatcgatatggccttcagcgtggtcgttggcttgggctcgggcaaaggccggcacgactacaacctcaagctcgacgcctcgggtagcctgatgtggctgcagtgcaagccctgcaatccgaagcagccacagcgcggccccctgttcgaccccaaggcctcgtccaccttccagcaggtcgccggcacgagccagatctgccacccgccgtaccccatggagcccgcggggcagcagtgcgccttccacctgtccggcgagcacggcatgtcggtgcacggcttcgtggccttggagaacctcaccatggggccagagtccatgaaggagttcgtcttcgggtgcgcgcactcggccgagcacttcaacagccagcgcaccttcgcgggcgtcgccgccatgggtaagatgcccacctccctcgtcatgcaggtggcggcgcgtgggcagacgcggttctcgtactgcctcttctccggcggggcgagccggcatggcttcctccggtttggcgccgacgtgccgagccggccgggcctccgaacgaccaagatcctcccggcgctggacgcgcacgagtcgcagtactacgtgagcctcgtgggcatcagcctggacgctaagaggctcacgcggatcaggccggagatgttcgcccggcggcgcggcgggcagggcgggtgcgtgatcgaccccggcacgccgctgacggtgctggcccgggaggcgtatcgcgtcgtggaggacgccgtctggagtgacctgcggcggaatagggccgagcgcatccagcggcagggctacgggttgtgcgtccgcaagaccgcggagatcaagcggcacctccagtcgctgtccttccacttcgcggaggagacggcgaggctggtcgtcaagccggaggagctgttcacggcggtggagggcaggctccacggtcccgccctgtgctttgccatgagcccgggcgagcggacggtcatcggcgcgctgcagcaggtggacacaaggttcgtgtacgacctaaaagacgctaaactgtcctttgcgtcggagccgtgttctcaggacaccgccggtgtggattga

SEQ ID NO: 6 - protein, 451 aa, Aegilops tauschii
  source 1..451: note = The sequence is a translation of the CDS of SEQ ID NO. 5
MAMAIKSTLQCVVFLMALITTHLIPPADADAGSPKVAMASSGAGSSFRLVAHHDYALRDDGFLHVQSRLDDLLPSEANVTTLRPPVASPIDMAFSVVVGLGSGKGRHDYNLKLDASGSLMWLQCKPCNPKQPQRGPLFDPKASSTFQQVAGTSQICHPPYPMEPAGQQCAFHLSGEHGMSVHGFVALENLTMGPESMKEFVFGCAHSAEHFNSQRTFAGVAAMGKMPTSLVMQVAARGQTRFSYCLFSGGASRHGFLRFGADVPSRPGLRTTKILPALDAHESQYYVSLVGISLDAKRLTRIRPEMFARRRGGQGGCVIDPGTPLTVLAREAYRVVEDAVWSDLRRNRAERIQRQGYGLCVRKTAEIKRHLQSLSFHFAEETARLVVKPEELFTAVEGRLHGPALCFAMSPGERTVIGALQQVDTRFVYDLKDAKLSFASEPCSQDTAGVD

SEQ ID NO: 7 - DNA, 1353 bp, Triticum aestivum
  source 1..1353: mol_type = genomic DNA
  CDS 1..1353: note = TaNep-1 gene encoding TaNEP1 aspartic protease
atggccatggccatcaagtccaccctccaatgcgtggtgttcctcatggccctcatcaccacccacctcatcccaccagccgacgccgacgccggctccccaaaggtggccatggcctcctccggcgccggctcctccttcaggctcgtggcccaccacgactacgccctcagggacgacggcttcctccacgtgcaatccaggctcgacgacctcctcccatccgaggccaacgtgaccaccctcaggccaccagtggcctccccaatcgacatggccttctccgtggtggtgggcctcggctccggcaagggcaggcacgactacaacctcaagctcgacgcctccggctccctcatgtggctccaatgcaagccatgcaacccaaagcaaccacaaaggggcccactcttcgacccaaaggcctcctccaccttccaacaagtggccggcacctcccaaatctgccacccaccatacccaatggagccagccggccaacaatgcgccttccacctctccggcgagcacggcatgtccgtgcacggcttcgtggccctcgagaacctcaccatgggcccagagtccatgaaggagttcgtgttcggctgcgcccactccgccgagcacttcaactcccaaaggaccttcgccggcgtggccgccatgggcaagatgccaacctccctcgtgatgcaagtggccgccaggggccaaaccaggttctcctactgcctcttctccggcggcgcctccaggcacggcttcctcaggttcggcgccgacgtgccatccaggccaggcctcaggaccaccaagatcctcccagccctcgacgcccacgagtcccaatactacgtgtccctcgtgggcatctccctcgacgccaagaggctcaccaggatcaggccagagatgttcgccaggaggaggggcggccaaggcggctgcgtgatcgacccaggcaccccactcaccgtgctcgccagggaggcctacagggtggtggaggacgccgtgtggtccgacctcaggaggaacagggccgagaggatccaaaggcaaggctacggcctctgcgtgaggaagaccgccgagatcaagaggcacctccaatccctctccttccacttcgccgaggagaccgccaggctcgtggtgaagccagaggagctcttcaccgccgtggagggcaggctccacggcccagccctctgcttcgccatgtccccaggcgagaggaccgtgatcggcgccctccaacaagtggacaccaggttcgtgtacgacctcaaggacgccaagctctccttcgcctccgagccatgctcccaagacaccgccggcgtggac

SEQ ID NO: 8 - protein, 451 aa, Triticum aestivum; identical to SEQ ID NO: 6
  source 1..451: note = The sequence is a translation of the CDS of SEQ ID NO. 7

SEQ ID NO: 9 - DNA, 1353 bp, Triticum aestivum
  source 1..1353: mol_type = genomic DNA
  CDS 1..1353: note = TaNep-1 gene encoding TaNEP1 aspartic protease
atggccatggccatcaagaacaccctccaatgcgtggtgttcctcatggccctcatcatgacccacctcatcccaccagccggcgccgacgccggctccccaaaggtggccatggcctcctccggcgccggctcctccttcaggctcgtggcccaccacgactacgccctcagggacgacggcttcctccaagtgcaatccaggctcgacgacctcctcccatccgaggccaacgtgaccaccctcaggccaccagtggcctccccaatcgacatggccttctccgtggtggtgggcctcggctccggcaagggcaggcacgaccacaacctcaagctcgacgcctccggctccctcatgtggctccaatgcaagccatgcaacccaaagcaaccacaaaggggcccactcttcgacccaaaggcctcctccaccttccaacaagtggccggcacctcccaaatctgccacccaccatacccaatggagccagccggccaacaatgcgccttccacctctccggcgagcacggcatgtccgtgcacggcttcgtggccctcgagaacctcaccatgggcccagagtccatgaaggagttcgtgttcggctgcgcccactccgccgagcacttcaactcccaaaggaccttcgccggcgtggccgccatgggcaagatgccaacctccctcgtgatgcaagtggccgccaggggccaaacccaattctcctactgcctcttctccggcggcgcctccaggcacggcttcctcaggttcggcgccgacgtgccaaggaggccaggcctcaggaccaccaagatcctcccagccctcgacgcccacgagtcccaatactacgtgtccctcgtgggcatctccctcgacgccaagaggctcaccggcatcaggccagagatgttcgccaggaggaggggcggccaaggcggctgcgtgatcgacccaggcaccccactcaccgtgctcgccagggaggcctacagggtggtggaggaggccatgtggtccgacctccaaaggaacagggccgagagggtgcaaaggcaaggctacggcctctgcgtgaggaagaccgccgagatcaagaggcacctccaatccctctccttccacttcgccgaggagaccgccaggctcgtggtgaagccagagcaactcttcaccgtggtggagtccaagctccacggcgccgccctctgcctcgccatgtccccaggcgagaggaccgtgatcggcgccctccaacaagtggacaccaggttcgtgtacgacctcaaggacgccaagctctccttcgcctccgagccatgctcccaagacaccgccggcgtggac

SEQ ID NO: 10 - protein, 451 aa, Triticum aestivum
  source 1..451: note = The sequence is a translation of the CDS of SEQ ID NO. 9
MAMAIKNTLQCVVFLMALIMTHLIPPAGADAGSPKVAMASSGAGSSFRLVAHHDYALRDDGFLQVQSRLDDLLPSEANVTTLRPPVASPIDMAFSVVVGLGSGKGRHDHNLKLDASGSLMWLQCKPCNPKQPQRGPLFDPKASSTFQQVAGTSQICHPPYPMEPAGQQCAFHLSGEHGMSVHGFVALENLTMGPESMKEFVFGCAHSAEHFNSQRTFAGVAAMGKMPTSLVMQVAARGQTQFSYCLFSGGASRHGFLRFGADVPRRPGLRTTKILPALDAHESQYYVSLVGISLDAKRLTGIRPEMFARRRGGQGGCVIDPGTPLTVLAREAYRVVEEAMWSDLQRNRAERVQRQGYGLCVRKTAEIKRHLQSLSFHFAEETARLVVKPEQLFTVVESKLHGAALCLAMSPGERTVIGALQQVDTRFVYDLKDAKLSFASEPCSQDTAGVD

SEQ ID NO: 11 - DNA, 1338 bp, Triticum urartu
  source 1..1338: mol_type = genomic DNA
  CDS 1..1338: note = TuNep-1 gene encoding TuNEP1 aspartic protease
atgggcatcaagaacaccctccaatgcgtggtgttcctcatggccctcatcatgacccacctcatcccaccagccgacgccgacgccggctccccaaaggtggtgatggcctcctccggcgccggctcctccttcaggctcgtggcccaccacgactacgccctcagggacgacggcttcctccaagtgcaatccaggctcgacgacctcctcccatccgaggccaacgtgaccaccctcaggccaccaatggcctccccaatcgacatggccttctccgtggtggtgggcctcggctccggcaagggcaggcacgactacaacctcaagctcgacgcctccggctccctcgtgtggctccaatgcaagccatgcaacccaaagcaaccacaaaggggcccactcttcgacccaaaggcctcctccaccttccaacaagtggccggcacctcccaaatctgccacccaccatacccaatggagccagccggccaacaatgctccttccacctctccggcgagcacggcatgtccgtgcacggcttcgtggccctcgagaacctcaccatgggcccagagtccatgaaggagctcgtgttcggctgcgcccactccaccgagcacttcaactcccaaaggaccttcgccggcgtggccgccatgggcaagatgccaacctccctcgtgatgcaagtggccgccaggggccaaacccaattctcctactgcctcttctccggcggcgcctccaggcacggcttcctcaggttcggcgccgacgtgccaaggaggccaggcctcaggaccaccaagatcctcccagccctcgacgcccacgagtcccaatactacgtgtccctcgtgggcatctccctcgacgccaagaggctcaccggcgtgaggccagagatgttcgccaggaggcacggcggccaaggcggctgcgtgatcgacccaggcaccccactcaccgtgctcgtgagggaggcctacagggtggtggaggaggccgtgtggtccgacctcaggaggaacagggccgagaggatgcaaaggcaaggctacggcctctgcgtgaggaagaccgtggagatcaagaggcacctccaatccctctccttccacttcgccgaggagaccgccaggctcgtggtgaagccagagcaactcttcaccgtggtggagtccaagctccacggcgccgccctctgcctcgccatgatcccaggcgagaggaccgtgatcggcgccctccaacaagtggacaccaggttcgtgtacgacctcaaggacgccaagctctccttcgtgtccgagccatgctcccaagacaccgcc

SEQ ID NO: 12 - protein, 446 aa, Triticum urartu
  source 1..446: note = The sequence is a translation of the CDS of SEQ ID NO. 11
MGIKNTLQCVVFLMALIMTHLIPPADADAGSPKVVMASSGAGSSFRLVAHHDYALRDDGFLQVQSRLDDLLPSEANVTTLRPPMASPIDMAFSVVVGLGSGKGRHDYNLKLDASGSLVWLQCKPCNPKQPQRGPLFDPKASSTFQQVAGTSQICHPPYPMEPAGQQCSFHLSGEHGMSVHGFVALENLTMGPESMKELVFGCAHSTEHFNSQRTFAGVAAMGKMPTSLVMQVAARGQTQFSYCLFSGGASRHGFLRFGADVPRRPGLRTTKILPALDAHESQYYVSLVGISLDAKRLTGVRPEMFARRHGGQGGCVIDPGTPLTVLVREAYRVVEEAVWSDLRRNRAERMQRQGYGLCVRKTVEIKRHLQSLSFHFAEETARLVVKPEQLFTVVESKLHGAALCLAMIPGERTVIGALQQVDTRFVYDLKDAKLSFVSEPCSQDTA

SEQ ID NO: 13 - DNA, 63 bp, Hordeum vulgare
  source 1..63: mol_type = genomic DNA
  CDS 1..63: note = Nucleotide sequence encoding a D-hordein signal peptide
atggctaagcggctggtcctctttgtggcggtaatcgtcgccctcgtggctctcaccaccgct

SEQ ID NO: 14 - protein, 21 aa, Hordeum vulgare
  source 1..21: note = The sequence is a translation of the CDS of SEQ ID NO. 13
MAKRLVLFVAVIVALVALTTA

SEQ ID NO: 15 - DNA, 60 bp, Hordeum vulgare
  source 1..60: mol_type = genomic DNA
  CDS 1..60: note = Nucleotide sequence encoding a C-hordein signal peptide
atgaagaccttcctcaccttcgtgctcctcgccatggtgatgtccatcgtgaccaccgcc

SEQ ID NO: 16 - protein, 20 aa, Hordeum vulgare
  source 1..20: note = The sequence is a translation of the CDS of SEQ ID NO. 15
MKTFLTFVLLAMVMSIVTTA

SEQ ID NO: 17 - DNA, 57 bp, Hordeum vulgare
  source 1..57: mol_type = genomic DNA
  CDS 1..57: note = Nucleotide sequence encoding a B-hordein signal peptide
atgaagaccttcctcgtgttcgccctcctcgtgatcgccgccacctccaccatcgcc

SEQ ID NO: 18 - protein, 19 aa, Hordeum vulgare
  source 1..19: note = The sequence is a translation of the CDS of SEQ ID NO. 17
MKTFLVFALLVIAATSTIA

SEQ ID NO: 19 - DNA, 63 bp, Triticum aestivum
  source 1..63: mol_type = genomic DNA
  CDS 1..63: note = Nucleotide sequence encoding a wheat glutenin signal peptide
atggccaagaggctcgtgctcttcgccgccgtggtgatcgccctcgtggccctcaccaccgcc

SEQ ID NO: 20 - protein, 21 aa, Triticum aestivum
  source 1..21: note = The sequence is a translation of the CDS of SEQ ID NO. 19
MAKRLVLFAAVVIALVALTTA

SEQ ID NO: 21 - DNA, 51 bp, Triticum aestivum
  source 1..51: mol_type = genomic DNA
  CDS 1..51: note = Nucleotide sequence encoding a wheat alpha gliadin signal peptide
atgaagaccttcctcatcctcgccctcgtggccaccaccgccaccaccgcc

SEQ ID NO: 22 - protein, 17 aa, Triticum aestivum
  source 1..17: note = The sequence is a translation of the CDS of SEQ ID NO. 21
MKTFLILALVATTATTA

SEQ ID NO: 23 - DNA, 87 bp, Hordeum vulgare
  source 1..87: mol_type = genomic DNA
  CDS 1..87: note = Nucleotide sequence encoding a HvNEP1 signal peptide
atggccatggccatcatgaacaccctccagtgcatcctcttcctcatggccctcatcatgacccaccagatcccgcgcgccaccgcc

SEQ ID NO: 24 - protein, 29 aa, Hordeum vulgare
  source 1..29: note = The sequence is a translation of the CDS of SEQ ID NO. 23
MAMAIMNTLQCILFLMALIMTHQIPRATA

SEQ ID NO: 25 - DNA, 435 bp, Hordeum vulgare
  regulatory 1..434: note = promoter - Promoter for D-hordein gene; regulatory_class = promoter
  source 1..435: mol_type = genomic DNA
cttcgagtgcccgccgatttgccagcaatggctaacagacacatattctgccaaaaccccagaacaataatcacttctcgtagatgaagagaacagaccaagatacaaacgtccacgcttcagcaaacagtaccccagaactaggattaagccgattacgcggctttagcagaccgtccaaaaaaactgttttgcaaagctccaattcctccttgcttatccaatttcttttgtgttggcaaactgcacttgtccaaccgattttgttcttcccgtgtttcttcttaggctaactaacacagccgtgcacatagccatggtccggaatcttcacctcgtccctataaaagcccagccaatctccacaatctcatcatcaccgagaacaccgagaaccacaaaactagagatcaattcattgacagtccaccgaga

SEQ ID NO: 26 - DNA, 431 bp, Hordeum vulgare
  regulatory 1..431: note = promoter - Promoter for C-hordein gene; regulatory_class = promoter
  source 1..431: mol_type = genomic DNA
aagcttacaaacttaatcccactcaagctatgcctatctcgatatgactacataaagtagagcatcacaaactaaattccaaaaagaggcaaaatctggattaatgtgtgtagtgtaaagtgaaaaaatgagtcatcattcattatcaagcatgccttacaacgagacgatatgtgcaacaaaaagcaactatgatgagcaatccaaaatcacacaagtaaagtagtactaccaaatacaacataccaaacgattagttgaataatcttaggagtactttttcaaaaagaaagggcaaggatgaaattataccataccatgacagctataaataaacatgcaccatcatggttgccctccatcatccaaactgcacacaccaagatcagaaacatcaattccaagaaagcaatagtaaccacaaatccaac

SEQ ID NO: 27 - DNA, 440 bp, Hordeum vulgare
  regulatory 1..440: note = promoter - Promoter for B-hordein gene; regulatory_class = promoter
  source 1..440: mol_type = genomic DNA
gtccacatgtaaagctttaacaacccacacattgattgcaacttagtcctacacaagttttccattcttgtttcaggctaacaacctatacaaggttccaaaatcatgcaaaagtgatgctaggttgataatgtgtgacatgtaaagtgaataaggtgagtcatgcataccaaacctcgggatttctatactttgtgtatgatcatatgcacaactaaaaggcaactttgattatcaattgaaaagtaccgcttgtagcttgtgcaacctaacacaatgtccaaaaatccatttgcaaaagcatccaaacacaattgttaaagctgttcaaacaaacaaagaagagatgaagcctggctactataaataggcaggtagtatagagatctacacaagcacaagcatcaaaaccaagaaacactagttaacaccaatccact

SEQ ID NO: 28 - DNA, 1922 bp, Triticum aestivum
  regulatory 1..1922: note = promoter - Promoter for wheat glutenin gene; regulatory_class = promoter
  source 1..1922: mol_type = genomic DNA
aaggtggcattggaggattgaggatgtttgtgttttttcttgtggggatgtctgcatttgttgttgaggtggattatgacaatctatcttttgcccattttattatttgttcaacattttatttgcttccatggctatctatttttgttgccgatacaatgaataaggttaataaagcataatttagcaaccacaaaatgtgtattaggagtcagggccgggccggcaaactcagggccctatgccaaaactctaacaatgagcctaccattagaagaacgtccggcaaagagatgcactgcaacatatgaccaaaacgtcatccatgatcgagtacaatttcttagtgcctttttcatcaaagttatatttgaaacattttagaaaatttgtcttaaattttttcccatggcgtttcgatcaaaaaaatgccttaaaacctacctatataaaggcaataagggaaaacacttcaggataccttcgaatctaaggtgtctttctttagatggtatgctaaactgttcttcatggcgcctcaaatcatcattctgcaagtaaagactaaaaataacgctaaatatggagttaaaggtttacaaacgacgagcggaaaaggagtcttatataattccagtagcatttattccattttgcttcacatagaaaatgtagctgaggtggtcgatgtttattttgactcgcgtgaggtcgccggttcgatctcagaagcaacgctggaatatcccatatagatttatttttcaggctgagtgatgctcgggtacctccagcgtatgggctgaaattcgccccccctgcaaatcatgggccctgtgacgttcgcacgggttgcacatgccttggcccgggcctactaggagtgtacctggattatgttggacgacgggagatgaaagggatgtattaattaacaaagataatgaagcttaattttcttatatgttgttaatattgacaagaaacaagctgctaactcaaagttacggttacatagtcgcaaccttttatatctaaataatatctctctctcaacatgcaaacatgccacctcagcatgtagcatgcatggaaaattgtccacttcaacatgcaaccatgcatcaaaatttccattttactaggctatttatttgataaaatttcacaaatatacaataatcaaacacaatagatcatatgtgttttcagttttggttctcacattattactccaaatataaatgtttcgtataaccaaatttcattcaaatatactgcaaaacatttccgtgaaaacatgtggggtacatctagttataaggaaatattagtgatgtcctgcaagtgataaggccaaggagagaagaagtgcaccatctacagaggccagggaaagacaatggacatgcagagaggcgggggcggggaagaaacacatggagatcatagaagaacataagaggttaaacataggaggaggatataatggacaattaaatccacattacctgaactcatttgggaagtggaaaaatcccctattctggtgtaaatcaaactaattgacgcgagttttctctgaagattctatgttaattttagacatgaatgaccaaaggtttcagttagttgagttttgtcatcgaaaggtgtttacataagtccaaaaattctaccagcttttggtacggcgcgtcatagaacagataaatgttgtgagtcattggatagatattatgagtcatagcatggatttgtgttgcctggaaatctaactatgacaagaaacaaaacataaatgggcttttgaaagatgatttatcaacttaccttatccatgcaagctaccttccactagtcgacatgcttagaagcttttagtgaccgcagatttgcaaaagcaatggctaacagacacc

SEQ ID NO: 29 - DNA, 593 bp, Triticum aestivum
  regulatory 1..593: note = promoter - Promoter for wheat alpha-gliadin gene; regulatory_class = promoter
  source 1..593: mol_type = genomic DNA
aagcttgtctagttacagtaacaacttgtggaacattacaaaatttatgtttgctagtaacttctagaacactacaacacttgacatgtataaggaatttgatgagtcatggcctactaaagcaagttatattactactcttatctatcttaacaggtcacacaagattacaaactaagttctgtatcagccatgcttatctagtttatgcataacaatttgcagaacattacaaacttagtttcggaaaaataggcaatctagattagtgtttgagctataaagtgaataagatgagtcatgcgtgttatcacacctctttggtggtggaatgatagtgcaacaacatgaaacttcagtgactagtccaagaatacacatgtaagtagtgccaccaaacacaacataccaaattatgattttgggaagcatccaagcactttccagacaagaaaatgccaattgtgaaagagatcataccatgggaactataaaaagccttgtagcatgatcatcatccttcctcacccatcattctcataagtagagcgcatcattcaagccaagcaagcagtggtcaatacaaatccacc

SEQ ID NO: 30 - DNA, 217 bp, Cauliflower mosaic virus
  regulatory 1..217: note = terminator - Nucleotide sequence of CaMV 35S terminator; regulatory_class = terminator
  source 1..217: mol_type = genomic DNA
ctagagtccgcaaaaatcaccagtctctctctacaaatctatctctctctatttttctccagaataatgtgtgagtagttcccagataagggaattagggttcttatagggtttcgctcatgtgttgagcatataagaaacccttagtatgtatttgtatttgtaaaatacttctatcaataaaatttctaattcctaaaaccaaaatccagtgacc

SEQ ID NO: 31 - DNA, 128 bp, Agrobacterium tumefaciens
  regulatory 1..128: note = terminator - Nucleotide sequence of Agrobacterium terminator; regulatory_class = terminator
  source 1..128: mol_type = genomic DNA
gaatcctgttgccggtcttgcgatgattatcatataatttctgttgggttacgttaagcatgtaataattaacatgtaatgcatgacgttatttatgagatgggtttttatgattagagtcccgcaat

SEQ ID NO: 32 - DNA, 1789 bp, Fusarium graminearium
  mRNA 1..1789: note = mRNA transcript TRI4 encoding trichodiene oxygenase
  source 1..1789: mol_type = genomic DNA
gtttcttttacaggtctatcaaagacttgagctttagaagatgattgaccaagattggatcaagagcttgctcaacatccccgtcagccatgttgctgggattttcgcagcatcgactgttatctacttcctctcttcctgcttttacaacctgtacttgcacccactgagaaagatcccgggaccaaagctcgctgccattggaccctaccttgagttctaccatgaagtcatccgggatggccaatatctctgggagatctccaagatgcacgataaatacggccccatcgtccgagtaaacgcccgcgaagttcacatcagggattcatcctactacactaccatctatactgctggttctcgcaagaccaacaaggaccccgccactgtcggtgcttttgacgttccctccgccactgccgccactgtcgatcatgaccatcatcgttctcgtcgcggctacctgaacccttacttctcgaagcgaaccatcaccaacctcgagcctttcatccatgagcgtgttaccaagcttttgactcgattccaacagcatctggacgacgaccaggtcctcagtcttgatggtgctttttgtgctttgaccgccgatgtcatcactaatcgattctatggcaagcacaacgactatctcagtcttcccgacttccactttgtcgttcgcgacggattcttgggtcttaccaagatctaccatcttgcacgcttcctccctggtctggtcaccattctgaagcgcctcccttactcttgtatccgcatgatcgcaccttctgtgtgtgatcttctccagatgcgagatgagattcaggaccgcggtggtgaggagttcctgtctaacaaatctcatgaggccaagtcatccatccttttcggtgcccttgcagactcgcacatcccctctcatgaacgaaccgtggagcgaatgctcgatgagggtaccgttatcctgtttgctggtactgagactacttcaaggacactggccattaccgtattatacctcttgacccatccagaatgtttgaaaaagctccgagaggagttgaacagcctcccacctgtcaaggacggccagtattctctcgctaccctagagaatctcccttacctgaacggtgtcatccatgagggattccgtcttgcttttggtcccatttctcgctcgggacgtgtggctactcaggagaacttgaagtacaaggagcatgtcatccctaaaggaactcccatttctcagtccacctatttcatgcacaccgatcccaagaatttccccgagcccgaaaagttcaagcctgagcgatggatcgaggcacaacagaagggtatccctctcaagaagtacatcaccaacttctctcagggttctagacagtgcatcggatacactatggcctttgctgagatgtacctcgccctttctcgcattgcgcgagcttacgacattgagctttatgacaccaccaaggccgacattgacatgactcacgcccgtattgttggctaccccaaggcaattccaggcaagaaggaacaccttggcgaagttcgagtcaaggttctcaaggctttgtaaggcgcatctgacaaactgtctcaatatcttactggataactcactgtatcggcatcgaatcctgttccttttgttcagtccatttttggtatgcaaggatggaaggtcatagtagcgacatctgaacgtaaaataaattgtaccctatttagacgctcgtcaatttaaacactattcatctcaggc

SEQ ID NO: 33 - DNA, 1309 bp, Fusarium graminearium
  mRNA 1..1309: note = mRNA transcript TRI5 encoding trichodiene synthase
  source 1..1309: mol_type = genomic DNA
ttattgaataactgttaccagtacaaccttgccatcatggaaaactttcccaccgagtattttctcaacactagcgtgcgccttctcgagtatattcgataccgagacagcaattacacccgagaggagcgcatcgagaatttgcactatgcttacaacaaggctgcccaccactttgctcagcctcgccaacagcagatgctcaaggtagaccctaagcgactacaggcttccctccaaacaatcgttggcatggttgtatacagctgggcaaaggtgtccaaagagtgcatggcggatctatctattcactacacctatactctcgttttggatgacagcagcgatgatccccatcctgccatgttgaactattttgacgaccttcaagccggacgagagcaggcccatccatggtgggcacttgtcaacgagcactttcccaacgtccttcgccattttggacctttctgctcattgaaccttatccgtagcactatggacttttttgagggatgttggattgagcagtacaactttggaggattcccaggatctgatgactaccctcaattccttcgtcgtatgaatggtttgggtcattgtgttggggcttctctatggcccaaggacctgtttgatgagcggaagcatttccttgaaatcacgtcagccgttgctcagatggagaactggatggtttgggtcaatgatctcatgtcattctacaaggaattcgacgatgagcgtgaccaaatcagtctggtcaagaactttgtcacctgccatgagatcactctggatgaagctttggagaagctcacccaggaaaccctacactcgtctaagcagatggttgctgtcttctcggacaaggaccctcaggtgatggacacgattgagtgtttcatgcatggctacgtcacgtggcacttgtgcgacgctcgataccgcctccatgagatttatgaaaaggtcaaggatcaggatacagaggacgccaagaagttctgcaagttctttgagcaggcggccaatgtcggcgccgttgcaccctcggagtgggcttatccacaagttgcacaactggcaaacgttcgggccaaggacgatgtgaaggaggctcagaagcccatcctaagttcaattgagctagtggagtaaccgaaggcgagtttggaagtatgttttgcgggtacggatactcgtttggagaatggtggtctgttataatgattacaaatagttcggtcgtgttttgttagaatgaacagttgaacaaggataattacttcggaataggcagttg

SEQ ID NO: 34 - DNA, 20 bp, Hordeum vulgare
  primer_bind 1..20: note = Fw Primer for HvNEP-1 transgene detection
  source 1..20: mol_type = genomic DNA
gcacttgtccaaccgatttt

SEQ ID NO: 35 - DNA, 20 bp, Hordeum vulgare
  primer_bind 1..20: note = Rv Primer for HvNEP-1 transgene detection
  source 1..20: mol_type = genomic DNA
cattgcctctggccccatgg

SEQ ID NO: 36 - protein, 508 aa, Hordeum vulgare
  PEPTIDE 1..508: note = H. vulgare phytepsin
MGTRGLALALLAAVLLLQTVLPAASEAEGLVRIALKKRPIDRNSRVATGLSGGEEQPLLSGANPLRSEEEGDIVALKNYMNAQYFGEIGVGTPPQKFTVIFDTGSSNLWVPSAKCYFSIACYLHSRYKAGASSTYKKNGKPAAIQYGTGSIAGYFSEDSVTVGDLVVKDQEFIEATKEPGITFLVAKFDGILGLGFKEISVGKAVPVWYKMIEQGLVSDPVFSFWLNRHVDEGEGGEIIFGGMDPKHYVGEHTYVPVTQKGYWQFDMGDVLVGGKSTGFCAGGCAAIADSGTSLLAGPTAIITEINEKIGAAGVVSQECKTIVSQYGQQILDLLLAETQPKKICSQVGLCTFDGTRGVSAGIRSVVDDEPVKSNGLRADPMCSACEMAVVWMQNQLAQNKTQDLILDYVNQLCNRLPSPMGESAVDCGSLGSMPDIEFTIGGKKFALKPEEYILKVGEGAAAQCISGFTAMDIPPPRGPLWILGDVFMGPYHTVFDYGKLRIGFAKAA

SEQ ID NO: 37 - protein, 437 aa, Nepenthes mirabilis
  PEPTIDE 1..437: note = NmNEP-1 aspartic endoprotease
MASSLYSFLLALSIVYIFVAPTHSTSRTALNHHHEPKVAGFQIMLEHVDSGKNLTKFELLERAVERGSRRLQRLEAMLNGPSGVETPVYAGDGEYLMNLSIGTPAQPFSAIMDTGSDLIWTQCQPCTQCFNQSTPIFNPQGSSSFSTLPCSSQLCQALQSPTCSNNSCQYTYGYGDGSETQGSMGTETLTFGSVSIPNITFGCGENNQGFGQGNGAGLVGMGRGPLSLPSQLDVTKFSYCMTPIGSSTSSTLLLGSLANSVTAGSPNTTLIESSQIPTFYYITLNGLSVGSTPLPIDPSVFKLNSNNGTGGIIIDSGTTLTYFADNAYQAVRQAFISQMNLSVVNGSSSGFDLCFQMPSDQSNLQIPTFVMHFDGGDLVLPSENYFISPSNGLICLAMGSSSQGMSIFGNIQQQNLLVVYDTGNSVVSFLFAQCGAS

SEQ ID NO: 38 - protein, 456 aa, Hordeum vulgare
  PEPTIDE 1..456: note = Hv aspartic endoprotease
MAGSHREGSKDRSGRKLLLVLLCGYYSGVAFAADDARTYKVLAVGSLKAEVVCSVTPASSSGTTVPLNHRYGPCSPAPSAKVPTILELLEHDQLRAKYIQRKLSGTDGLQPLDLTVPTTLGSALDTMEYVITVGIGSPAVTQTMMIDTGSDVSWVRCNSTDGLTLFDPSKSTTYAPFSCSSAACAQLGNNGDGCSNSGCQYRVQYGDGSNTTGTYSSDTLALSASDTVTDFHFGCSHHEEDFDGEKIDGLMGLGGDAQSLVSQTAATYGKSFSYCLPPTNRTSGFLTFGAPNGTSGGFVTTPMLRWPKAPTLYGVLLQDISVGGTPLGIQPSVLSNGSVMDSGTVITWLPRRAYSALSSAFRSSMTRLRHQRAAPLGILDTCYDFTGLVNVSIPAVSLVLDGGAVVDLDGNGIMIQDCLAFAATSGDSIIGNVQQRTFEVLHDVGQGVFGFRSGAC

SEQ ID NO: 39 - protein, 6 aa, synthetic construct
  PEPTIDE 1..6: note = SEKDEL tag
SEKDEL

SEQ ID NO: 40 - DNA, 2500 bp, Hordeum vulgare
  regulatory 1..2500: note = promoter - Hordeum vulgare promoter for HvNEP1 gene; regulatory_class = promoter
  source 1..2500: mol_type = genomic DNA
ctacagcatcatatgtagtgaagtcgggtgtgctttcctcgatgctagattgtgagaactcagtggcatgttctttagaggaagtgtgaatgctttcttccatccttgattgtgagaaatcagtggcatcttttgatactggcacaagttgtagaggactagagacacactgctgctgattttatctgaagcaacagctccagcatcactgactgtatcttttgatagcgcttgtagatgaatcggttcaagtattaccataatctacgttgcgcaaagctgtgggcctgccaggggcatcttgatctttcaatacgctgaccacctctacaggcataagtacagtaccatctgcattactgaaagtcagagctactgtgtcttcattgctctctagctttgtctgatgttgcaaattttgtgacaacttctctctagcttccaaaatctgtgccaagtaaaaaaaaggatataagaaattcaccaccaaaaaaaggtaataccaccaacttctctattgtgcaaccattaacattttaagcattgacctcagtcaataaatttatttatcaagcaagaatatgaacactaaaatatcttaaactactactcattccgtcccaaaataagtgtcttgagcttagtacaactttatactagagctagtatatagttcagacacttattttgagacggaggaagtattacacattagtttgaaaatcagcactttttagtttcattgtgaaaagacaatgttccaatatttgtacagcccgtttagtaatttagtatgctagcaaaaatttccaaatgggtaaatttagaagccaaaccaagtgttggcatcgcaaagtttgtggctagtcaagttttggcatcgcaaatgttggtagcaaacaaagaagactcgtagtgacacaaccctcactgtcatgcacatcaacatgatgttcaataacatctacatcaaagtcttctccatgatatatccaacaagtatatgtactttccatgccatactcaatatgtgcgtgttcgcaacggtctgatgcttgtacatatgattaagatgtttttcttttacatgatcagagcatttaatcatcctcgttgattttctcttgaatgaagttcataaattctttgacacattagatgtagatataattaaaattcgttcattaatttggaaaagtttgcgaattttaaataattacatggcacacgggataaccagaagaaaacacggcgagaccaaataaaagtttacacgaatcttggagtgattaatcgtgtggtacatgacttagatgtgcaatacttaaatctcatctagatgtagctttggaaaaggaatacactatctatcggtctttttttataaaggacgtttttattaactcataacataggatcaaaaggatacaaataatgacagggttacgacccgtgggaacgacaaaacgaaggaaaccccactccaaaacgtttgagggtgggctgccccctgggccagctggcggcaggcggcccgtcttgccgtcatgctgctggccggcccgtccagctggccccgacagcagccggtgggtcagcgcccgtcccatccgcatttggaaaaattgttagtgtacctaaaaagtgatcacgaatttttaaagaattcacgcatttgaaaaacattcacaaaataaaaaaagttcatgatcctgaataaaaagttcatagatttgaaaagaatttgcgaatttgaaaaaagttcatgaatttgaaaacagttcgtgaatatgaaaaacatttacacattttaaaaaggttcatgaacttgaataaaaaggtcaaggatttgaaaaaagtttgcgcatttgaaaaatattcatgatttaaaaaaaacgttcatgcatttgaaaaacattctcgaattcgaaaaaaaatcaggaacatgaatgaaaagttcacggaatagaaaaatgtttgcacatttaaaaatgctcatgaatttggaaaaaagtcacagatatgaaaaatgttcgtgaatttgaaaaaaattcatgaacttgaatgaaaagtttacagaactgaaaaacgtccatgaattcgaaaaagttcgcaaatttttgaaaagtagaggacacgcgggacaacaaaaaaacacactgcaaacgattaatcgcgtagtacatgacttaaatgtgtaatacttaaatctcatgtagatgtatcttagcaaaaggaatgcaatactatatattgtctacacatccttaagctgttatagtgacatcaaatatgatctagacatccttaagcacatctttaagctgatgtactaggtcaaatagtgccatggtgatcactgccatatctccaattcgagcttcagtagcccaaagatatgcaaattaagtcagatcagagtggtggtagatgtgctatataaacgtgatgagtatattcctccatccaaggccacatcccacacataattagcacatca

SEQ ID NO: 41 - DNA, 787 bp, Hordeum vulgare
  regulatory 1..787: note = promoter - Hordeum vulgare promoter for HvLTP1 gene; regulatory_class = promoter
  source 1..787: mol_type = genomic DNA
gagctccaaggcatcaccaagcttctatgacgccaaaacatccaagaaagatatgtactaggataccaagcacccaagagtaaacggaggaagtataatataaggccctgtttgataacaaagtagtaaaaaaactaaagtattaaaaactgcagtaattttacgtgtagatagaaaataccatggttttaatataataatattttttgcagtattcacaatgtagagaaactgtttgattacgccacatattactgcagtttagatcgagcaagtacacgggaagaagataacgacgtcccaccccttcttttcgccttctctgttttttaaaaagaggtctggggttagttttttcaatactgcagttttaaaatcacaattcttagaggcaaccaaacacctcattgtaaataaaactatgataatctccaaaactgcagtattctaaaaatactacaaaaattctttgttatcaaacagggcctaaggagttaaaaaaatttagccgtaactgagactcggcgaggcaccagcagctagcagtcatcaacacttgatggttggcaaaggcgagtcgacgtgtcgcggggctcggcctgagcgggagatacaatctgttctccagtaaccccgtcgatttggcccgccgactaaagcatccaggcatctctcgctcgaacccctatttaagcccctccattcctcccaacattctccacacctccacgagttgctcatcactagctagtacgttgtactgttagctacagattaagaagtgatc

SEQ ID NO: 42 - protein, 4 aa, synthetic construct
  PEPTIDE 1..4: note = KDEL tag peptide
KDEL

SEQ ID NO: 43 - protein, 4 aa, synthetic construct
  PEPTIDE 1..4: note = HDEL-tag peptide
HDEL

SEQ ID NO: 44 - DNA, 1898 bp, Zea mays
  source 1..1898: mol_type = genomic DNA
  CDS 422..1783: note = ZmNEP-1 gene encoding ZmNEP-1 having protein ID: XP_008668084.1
cttttttatttctccatctccatgctccgatgccgctgatgatcttgccaacagaggtggaaaattgcagtcaatggatacctgcacggcggttctattctgtagaacgttcttctgattatgctgctgctgcttgctcaaaaaagtgcctaacaattatccaacaacgaccccagccaggcccacgttgaatttagtagaagcatgtttgaacccttattgcccgcacgccgaacaaagaggtcacctaaccacttaaaaattcagcgcccatacaaccgtaggcgccatcttcttggcgtgagcgcgacaacaatgctagcgagcgctgcagactgtttcatctcttccaggcaactcaccagctgagactgagaccggcacaagatggcggctctgaccagccagccaccatagctccatgtcgtcgtcgacctcacaaatggcgtcgctcgccgtgctcgtcttcctggtggtctgcgcaacgcttgcgtccggtgccgccagcgtccgcgttgggctcacgcgcatccactccgacccggacaccaccgcgccccagttcgtgcgcgacgcgctgcgccgcgacatgcaccggcagcggtcccgatcgttcggccgcgaccgcgaccgcgagctcgcggagtccgacgggcgcaccacggtgtccgcgcgcacccgcaaggacctgcccaacggcggggagtacctcatgacgctggccatcggcacgccgccgctgccgtacgcggccgtcgccgacacgggcagcgacctcatctggacgcagtgcgcgccctgcggcacccagtgcttcgagcagccggcgccgctgtacaacccagcgagctcgaccacgttcagcgtgctcccgtgcaacagctccctgagcatgtgcgcgggggcgctggcgggggccgcgccgccgcccgggtgcgcctgcatgtacaaccagacgtacggcaccgggtggacggcgggcgtgcagggctccgagaccttcaccttcggctcgtccgccgccgaccaggcccgcgtccccggcgtcgccttcggctgcagcaacgccagcagcagcgactggaacggctcggcggggctggtggggctgggcaggggcagcctgtcgctcgtctcgcagctcggcgccggcaggttctcctactgcctgacgccgttccaggacaccaacagcaccagcaccctcctcctcggcccgtcggcggcgctcaacggcaccggcgtccgctccacgccgttcgtcgctagcccggccagggcgcccatgagcacctactactacctcaacctgacgggcatatccctgggcgcgaaggcgctgcccatctctcccggcgcattctccctcaagcccgacggcacgggcggcctcatcatcgactccggcacgaccatcacctcgctggccaacgcggcgtaccagcaggtccgcgccgcggtaaagtccctggtcacgacgctgccaacggtcgacgggtcggactccacggggctcgacctgtgcttcgcgctgccggccccgacgtcggcgccgccggccgtgctgccgagcatgacgctccacttcgacggcgccgacatggtgctccccgcggacagctacatgatctcggggtccggcgtgtggtgcctggccatgcggaaccagacggacggcgcgatgagcacgttcgggaactaccagcagcagaacatgcacatcctctacgacgtccgggaggagacgctgtcgttcgctccggccaagtgcagcactctttgacgatgcgatagttgtacatatgtatatgtgtgcatatataggattcatgattttttttgtatacagtggattgttaaccgaacacactaattaattccattattgttgactgcta

SEQ ID NO: 45 - protein, 453 aa, Zea mays
  source 1..453: note = The sequence is a translation of the CDS of SEQ ID NO. 44
MSSSTSQMASLAVLVFLVVCATLASGAASVRVGLTRIHSDPDTTAPQFVRDALRRDMHRQRSRSFGRDRDRELAESDGRTTVSARTRKDLPNGGEYLMTLAIGTPPLPYAAVADTGSDLIWTQCAPCGTQCFEQPAPLYNPASSTTFSVLPCNSSLSMCAGALAGAAPPPGCACMYNQTYGTGWTAGVQGSETFTFGSSAADQARVPGVAFGCSNASSSDWNGSAGLVGLGRGSLSLVSQLGAGRFSYCLTPFQDTNSTSTLLLGPSAALNGTGVRSTPFVASPARAPMSTYYYLNLTGISLGAKALPISPGAFSLKPDGTGGLIIDSGTTITSLANAAYQQVRAAVKSLVTTLPTVDGSDSTGLDLCFALPAPTSAPPAVLPSMTLHFDGADMVLPADSYMISGSGVWCLAMRNQTDGAMSTFGNYQQQNMHILYDVREETLSFAPAKCSTL

SEQ ID NO: 46 - DNA, 1943 bp, Glycine max
  source 1..1943: mol_type = genomic DNA
  CDS 426..1787: note = GmNEP-1 gene encoding GmNEP-1 with protein ID: XP_003523200.1
attgccttagatacgttttgcaacaaataataaaatctttaccaacctcaacgcaagactcggtacttaattgttgcgacactacgctgataccttaacctccattcatcatcaaacacacgacgtttctctgttcacaccaaaacaaaacttctctctctctgtctccccttttgtttttttccttcaaagaaaaatttgacaagccaaaactccccttcttgcttcttcccttaatcctctccaccacattcgaagggaacgttacaaaaaaatctccattttttctcaagttaatcaagtaagataagatcattcccctctatcaacaaacctttattcttatatatacattcccacaattcccatcactcattcattccactttatataatttcccctccactccacattgtgcacccttcatggtcatggcaaaactaaaacacccttcatcttttgtcacattggtggcacttcttctagcagtgtctcttttcgttgctccaacatcctcaacatccagaaaaactattctcaagcaccacccttacccaacaaaagggttccgagtcatgcttcgccacgttgattcgggtaaaaatttaaccaaactagagcgtgtccaacacgggatcaagcgtgggaagagtaggcttcagaggcttaatgcaatggtgttggcagcatcaacactagattctgaagatcaattagaagcccctattcatgcagggaatggagaatatttaatggagttagccattggaaccccaccagtgtcttaccctgcggttttggacactggcagtgaccttatttggacacagtgcaagccttgcacgcagtgttataaacaaccaacacccatttttgatcccaagaagtcctcttctttttccaaggtttcatgtggtagcagcttgtgcagtgctgtgccttcttcaacatgcagtgatgggtgtgagtatgtttattcatacggtgactattcaatgacacaaggcgttttggccactgagactttcacttttgggaagtctaagaacaaagtttcggttcacaacattggttttggttgtggggaggacaatgaaggtgatggatttgaacaagcttcagggttggttggtcttggacgtggtcctttgtccttggtttctcaactcaaggaaccgagattttcttattgtttgaccccaatggatgacacaaaagaaagtattttgttgttggggtctttgggtaaagtgaaagatgcaaaagaagtggtgacaacacctcttctcaaaaaccctttgcaaccttctttttactatctttctcttgaaggcatctctgttggggacactcgattgtccattgagaagtccacttttgaagtgggggatgatgggaatggtggtgtgatcatagactctggcaccacaatcacctacattgaacaaaaggcctttgaggcactcaaaaaagagttcatttctcaaaccaaacttcctttggacaaaactagctcaacagggttggatctttgcttctctctgccatcagggtcaacacaagtggagattccaaagattgttttccatttcaagggtggggatttggagcttcctgctgagaactacatgattggtgactccaatttgggtgtggcttgtttagccatgggtgcttctagtggaatgtctatattcggaaatgttcaacagcagaacattttggtgaatcatgatcttgaaaaggagaccatttcttttgttcctacgtcgtgtgatcagctgtgagtgtgtgatattcactatatgtttttattgctttgtttgtttgatgatgttctgttgccgaactcgtattgctatgattgaatctcttagttgttgcaataatatgaacattttattctctgtccaattcaaatggatcagcacattaatagaaca

SEQ ID NO: 47 - protein, 453 aa, Glycine max
  source 1..453: note = The sequence is a translation of the CDS of SEQ ID NO. 46
MVMAKLKHPSSFVTLVALLLAVSLFVAPTSSTSRKTILKHHPYPTKGFRVMLRHVDSGKNLTKLERVQHGIKRGKSRLQRLNAMVLAASTLDSEDQLEAPIHAGNGEYLMELAIGTPPVSYPAVLDTGSDLIWTQCKPCTQCYKQPTPIFDPKKSSSFSKVSCGSSLCSAVPSSTCSDGCEYVYSYGDYSMTQGVLATETFTFGKSKNKVSVHNIGFGCGEDNEGDGFEQASGLVGLGRGPLSLVSQLKEPRFSYCLTPMDDTKESILLLGSLGKVKDAKEVVTTPLLKNPLQPSFYYLSLEGISVGDTRLSIEKSTFEVGDDGNGGVIIDSGTTITYIEQKAFEALKKEFISQTKLPLDKTSSTGLDLCFSLPSGSTQVEIPKIVFHFKGGDLELPAENYMIGDSNLGVACLAMGASSGMSIFGNVQQQNILVNHDLEKETISFVPTSCDQL

SEQ ID NO: 48 - DNA, 1383 bp, Gossypium hirsutum
  source 1..1383: mol_type = genomic DNA
  CDS 1..1383: note = GhNEP-1 gene encoding GhNEP-1 with protein ID: XP_016704203.1
atgtctttatcccttcgttttctcagcgctaaactgttcttatgcctctgtttaacattatttcaacaccatgtcacgttttctgcttcgaatcctactggtctaaccctaagggctgtcctggatgattctccaaactctcctttataccttattgaaaacatgactatagctgaaagaatcgaaagatttatccaagttaccaatgctaaagacaattatttgaatcttaatgcaagggtaggccctgataattctaattctctatctcgagtagtaatggctcgagatggtttattttattcagtatggcttctaataggaagccaaggccaagaagtgaagctgttgatggacacaggcggtggtctaacatggacgcagtgtcagccttgcctaaattgtttcccacagaatcttccaatttatgattctagaacttccactacttactccactctttcttgtgaccatcctctctgccaagtcgagggtagcctttatacttgtgtcgatgacttatgtatcttcgttcataattatcatggcggcctctacactacgggggtcgcatccctggaaacattctatttccctatggacccatctactgctctaactttcaataatctggtcttcggttgctctcgggatagtcgtaacgttgtttttcaggacaccgaactttcagggatctttggaatgaacatgatgccggattcattgatgagtcagctttctagttttactaactttcgattctcctactgtttggtcccatttcctgatttaatacctcatacacttgttctaaggttcggagatgacattccactgttgcctccagaacgtgttaaaacaacgatgttcgtgcacgcaccttacctctataattactacgtgaacctggtgacaatcagttttctaaatgatcgtctaggatttcctccatctcaatttcagctgagggaagacggattaggtggttgcttcgttgactctggatatttgctcaccgcaatcgaagacaactatgttggaggggtgaatgcatatgatgtactaatggatctgtttacagcttattatgagagcaacaatcttagaagaacaacggatccgtcaggacttgacatgtgttttgaacgtccaaatgattttaataattttgcaaatctaacattccattttgatggtgaagccgattacttcgttcctccacagcatttgcatatcttccaacaagatcacttctgcgtagcaataacaaggggaagatacgcaactgtgcttggagcatggcagcaacaaaataaacgtatgctttatgatgtagggcttggtagactccaatttgctgatgaaaactgtgcgaatgattaa

SEQ ID NO: 49 - protein, 460 aa, Gossypium hirsutum
  source 1..460: note = The sequence is a translation of the CDS of SEQ ID NO. 48
MSLSLRFLSAKLFLCLCLTLFQHHVTFSASNPTGLTLRAVLDDSPNSPLYLIENMTIAERIERFIQVTNAKDNYLNLNARVGPDNSNSLSRVVMARDGLFYSVWLLIGSQGQEVKLLMDTGGGLTWTQCQPCLNCFPQNLPIYDSRTSTTYSTLSCDHPLCQVEGSLYTCVDDLCIFVHNYHGGLYTTGVASLETFYFPMDPSTALTFNNLVFGCSRDSRNVVFQDTELSGIFGMNMMPDSLMSQLSSFTNFRFSYCLVPFPDLIPHTLVLRFGDDIPLLPPERVKTTMFVHAPYLYNYYVNLVTISFLNDRLGFPPSQFQLREDGLGGCFVDSGYLLTAIEDNYVGGVNAYDVLMDLFTAYYESNNLRRTTDPSGLDMCFERPNDFNNFANLTFHFDGEADYFVPPQHLHIFQQDHFCVAITRGRYATVLGAWQQQNKRMLYDVGLGRLQFADENCAND

SEQ ID NO: 50 - DNA, 251 bp, Zea mays
  regulatory 1..251: note = promoter - a-Zein gene promoter; regulatory_class = promoter
  source 1..251: mol_type = genomic DNA
gcattacaaagttagcttcacaagcgtatgaattcattgacaacccttgacatgtaaagttgattcatatgtataagaaagcttaatgatctatctgtacatccaaatccatgtactatgtttccacgtcatgcaacgcaacattccaaaaccatggatcatctataaatggctagctcccacatatgaactagtctctatcatcatccaatccagatcagcaaagcggcagtgcgtagagaggatcgtcg

SEQ ID NO: 51 - DNA, 2335 bp, Oryza sativa
  regulatory 1..2335: note = promoter - glutelin GluB-1 promoter; regulatory_class = promoter
  source 1..2335: mol_type = genomic DNA
acagattcttgctaccaacaacttcacaaagtagtagtcaaccaaaactatgctaaggaatcacctcacttccgcccatgaccgtgagcacgactgttcaaacagtttgttaatctctacaaagaaggtacactttacctacacaacgccactaacctgagttacccagcccatgcaaaatagccacgtcttgtgacttaagggatttcgcgacaaggcatttcgaaagcccacacaaggacaccttatgaaaactggaggggtcccacagaccaacaacaagttaggtcccaaaccatgttgtgccaggaaaaatccaaggggtcctccccaacaccaccccgacaaatccacttgtccattggcatcaagatttgcctgacctagctaattactcagccaggcatgtcacaattcacccatgtggtcacacatgttaggttggagaaattctaaaggaaaggaatcggtccatatgagcaagaccgagaaaccataccaccagtacttctaccgaaatacgagtttagtaaactcatttgttttcaaggcacccgacccaggtgtgtcgggttttccagggattttgtaaacccaagttttacccatagttgatcattcaaattttgaggagggtcattggtatccgtacctgagggcacgaatactgagacctagcattgtagtcgaccaaggaggttaatgcagcaattgtaggtggggcctgttggttatattgcaaactgcggccaacatttcatgtgtaatttagagatgtgcattttgagaaatgaaatacttagtttcaaattatgggctcaaataatgaaaggtgacctaccttgcttgatatcttgagcttcttcctcgtattccgcgcactaggagatcttctggctccgaagctacacgtggaacgagataactcaacaaaacgaccaaggaaaagctcgtattagtgagtactaagtgtgccactgaatagatctcgatttttgaggaattttagaagttgaacagagtcaatcgaacagacagttgaagagatatggattttctaagattaattgattctctgtataaagaaaaaaagtattattgaattaaatggaaaaagaaaaaggaaaaaggggatggcttctgctttttgggctgaaggcggcgtgtggccagcgtgctgcgtgcggacagcgagcgaacacacgacggagcagctacgacgaacgggggaccgagtggaccggacgaggatgtggcctaggacgagtgcacaaggctagtggactcggtccccgcgcggtatcccgagtggtccactgtctgcaaacacgattcacatagagcgggcagacgcgggagccgtcctaggtgcaccggaagcaaatccgtcgcctgggtggatttgagtgacacggcccacgtgtagcctcacagctctccgtggtcagatgtgtaaaattatcataatatgtgtttttcaaatagttaaataatatatataggcaagttatatgggtcaataagcagtaaaaaggcttatgacatggtaaaattacttacaccaatatgccttactgtctgatatattttacatgacaacaaagttacaagtacgtcatttaaaaatacaagttacttatcaattgtagtgtatcaagtaaatgacaacaaacctacaaatttgctattttgaaggaacacttaaaaaaatcaataggcaagttatatagtcaataaactgcaagaaggcttatgacatggaaaaattacatacaccaatatgctttattgtccggtatattttacaagacaacaaagttataagtatgtcatttaaaaatacaagttacttatcaattgtcaagtaaatgaaaacaaacctacaaatttgttattttgaaggaacacctaaattatcaaatatagcttgctacgcaaaatgacaacatgcttacaagttattatcatcttaaagttagactcatcttctcaagcataagagctttatggtgcaaaaacaaatataatgacaaggcaaagatacatacatattaagagtatggacagacatttctttaacaaactccatttgtattactccaaaagcaccagaagtttgtcatggctgagtcatgaaatgtatagttcaatcttgcaaagttgcctttccttttgtactgtgttttaacactacaagccatatattgtctgtacgtgcaacaaactatatcaccatgtatcccaagatgcttttttattgctatataaactagcttggtctgtctttgaactcacatcaattagcttaagtttccataagcaagtacaaatagct

SEQ ID NO: 52 - DNA, 1381 bp, Glycine max
  regulatory 1..1381: note = promoter - G. max b-conglycinin promoter; regulatory_class = promoter
  source 1..1381: mol_type = genomic DNA
agtgcttggatttggaccagacttgaattttaatttaatgatattataatatgtgaatatatttttgagacaattgtaaatttcagataaaaaaataatgtaattaaaattgtaataactatatcgtatacttaattaattattaaatgtgacaaaaaagatatacatcaaaacttaatgtttcatgacttttttttaatgtgtgtcctaaatagaaattaaaaataaaaattattatatccaaatgaaaaaaacatttaatacgtattatttaagaaataacaatatatttatattttaatatgtattcacatgtaaatttaaaaacaaaaacaaaatttctcttttattgattaattaaaataattttataactacatttattttctattattatcaattttcttctgtttttttatttggcatatatacctagacaagtcaaaaaatgactattctttaataatcaatcattattcttacatattggttttcgaactacgagttatgaagtgttccaattgcaccttagtgtttttgataggccttccccatttgccgctcattaattaatttgataacagccgtaccccgatcaaattactttatgcttcttcccatcgtaaattatatgcatgtcgggttcttttaatcttggtactctcgaattggccaccacaaccactgactagtctcttggatcatgagaaaaagccaaagaacaaaaaagacaacataaagagtatcctttgcaaaaaaaatgtctaaagttcataaaatacaagcaaaaacgcaatcacacacagtggacccaaaagccatgcacaacaacacgtactcaccaaggtgcaatcgtgctgcccaaaaacattcaccaactcaatccatgatgagcccacacatttgttgtttgtaaccaaatctcaaacgcggtgttctctttggaaagcaaccatatcagcatatcacactatctagtctcttggatcatgcatgcgcaaccaaaagacaacacataaagtatcctttcgaaagcaatgtccaagtccatcaaataaaattgagacaaaatgcaacctcaccccacttcactatccatggctgatcaagatcgccgcgtccatgtaggtctaaatgccatgcacatcaacacgtactcaacatgcagcccaaattgctcaccatcgctcaacacatttcttgttaatttctaagtacactgcctatgcgactctaactcgatcacaaccatcttccgtcacatcaattttgttcaattcaacacccgtcaacttgcatgccaccccatgcatgcaagttaacaagagctatatctcttctatgactataaatacccgcaatctcggtccaggttttcatc

SEQ ID NO: 53 - DNA, 1650 bp, Glycine max
  regulatory 1..1650: note = promoter - G.max soyAP1 promoter; regulatory_class = promoter
  source 1..1650: mol_type = genomic DNA
agtggagtagcaaaggacgagaggtaggggtgtagggaaattgccaacagggtagttttgggagtaagaattttgggagtgataatagcaaccctcaagtaagtcctttagcagaccaaacactaaaaatacaaacgaataaacatctaatgggccttagactcaggcttaaattgaagaaccatacatgtcagtgtcaccctgcaaaaaaggtgagaactgagaactattacaaaattgttatatgactgcatgctgagatttattaaattcttaaccgaccttaaaactcttatgtaaatgtgttttttcagcgtgattttttttattttcaatttattttaatattctaaaaatcatcaagttctatgattacttttttttaatatcaaatattaaatttattgatgaaaggaaaattcaattgaatccctttaaacatagtttggaatatccttaaaaacatgatttgtgaagattggaagataatttaacaaaaagtataaatgtataataggaaatgaaggtgtaactgtgtaagtgaagacaagcataaaagagaaatgaggagagggaggtgaggtgtcgcgtgctaaggaagccaagtggtgcagatgctggcatcgttttctagttttaagggattctgttgcaaaccccactcgctacgtatctgcatgcatgatgcatatgcatatgcatggtctcagggtaaaccgttcctttttcttcattcatctttaccaacccatcctttcatatctacggccaagatcacgtagaaatggacggtgatgattgaaagattgcaccgccaagtttatttgttgttttaggggaatttggcctgcgttgcgttcttattaggcgagaagaaaggaataaaggggaaggaaggtgtgacactactgtcatactgcactgcttacaacttttttctctttctctcaattcaattgccttctcccctgcgaatctcttctccacgtatcggtaaacctattcctctaacccccattctcattctttcatcgcattttactttattcatcttaaacagccctcagtctctcatctgttttcctaaccgcgtttcattttttatttattttgtttttatgcgcagattgtccctgcaaattgcactttataatataaataatcgctttttattttctgtttatgtcaggcgaattcaattttttttcttttgcttcccttgtttcggtggataacaaaaaaaaaataaaatctattatcgaggtctctttttcaaattgcacggatgcgtcgattttttttcgataaaaaaaaatccatatcggtatgatcgaacacatgatattttttttcgttcgtataccattcggtgatttttttttataatttttcacaactcaattttcttgttttgtttgcattggtttttgtggaatagactatttttttgactgaaatggtggaatagactatagagattagaagaactgacacaagattttgaaatgtctcgtttttttttcacgtccccataataatatatttagcattttcacttgttagttaaagcccacatcccctaatttagagtaattatttatgtgctaacaattgcaattaaagtttatttatttggatgaataggagaac

SEQ ID NO: 54 - DNA, 1138 bp, Gossypium hirsutum
  regulatory 1..1138: note = promoter - G. hirsutum a-globulin A promoter; regulatory_class = promoter
  source 1..1138: mol_type = genomic DNA
ctattttcatcctatttagaaatccaagttgacacctaaaatttagttggactgccatgtaggattatcgttagagagataacggagcttaacggtagagtgatcactttgtaacaaaataataacaaaagtgactaaagtgtaacatttcaaacataaatgattaaaatataacctgaggcaaacaaaaatgactatttttatagattaccctaaaattaaagagtcatggccctagcccctcgcctacttgtttgtttttaataaactaacatagtataatatattgttaggattatataaaattattaataaatagtataattaatttaaaatttatgaaaaataaattaccatatttcttaaatacgtggcaccttatgttggattggactgtataacttatatactattatctatattgaatccaaatccttacttttaagcgtttttagtgaaacattttattttccattcttattatataaatttatataatgatataatatgtaatacttagataatattattgaaaaagaataaaaatacctcaaactttgaaaggactaatttgtatgagcatcaaacgtacaggataccaaaagtatacatatctgaatttgttcatatctcctgcaactcatagatcatcaccatgcacatgtgtacacttgacttgtcctctatcaactcaacccttaactcagtgaatcgggacatctctgtctcactttaaaacccttcccagtttcaacactctttgaattcaactgagttcacatacaacacaacacagtccatcatctttctgctgttaaagcatcatcatttcgccccttccagttacagatgcaacatgaccccccctgcaacaaagtttgtccgaaccttgctagtaccatgtgaagggatgtggcatctcgatatctacccaccactatacaaaaaaaaaaaaaagagacaatatttcgtcttctttaatttgcacactcgtcatcttgcatgtcaatgtcttcaacacgttgatgaagatttgcatgcaaaaatatcaccttccacagctccaccttctataaatacattaccactctttgctattaccatcacacagtaacaaaatacagagcttatcgtaatc

SEQ ID NO: 55 - DNA, 1227 bp, Gossypium hirsutum
  regulatory 1..1227: note = promoter - G. hirsutum storage protein (Gh- sp) promoter; regulatory_class = promoter
  source 1..1227: mol_type = genomic DNA
caatcaagattttcagaaccaggtcgatagttgaattagttatgttattggtccgactagtttgattaaaaattattaaaaattcataaaataagaatagaaaaatcgctctaatcaagttttttagttcgacaagtaccaattcatggatcaacctgcttaacctcttgttttggacaatacctcaaccgcttcttgatccaatcggttcggatcactaaaatacccctagaaggagatgaggctaagcagagcgaaaataactttccacgagacgagaatggaaactattgtatttaaatattttgattggattcaacaatcaatattttgtaaaggtaagtatttccataaactatttaagaataatgattcttcatgtgcagaacgcggcggtactattttcaagatacaatacattactcgacggaacaattcgtattgcagtaccaattattttaaactgaatgaaatttagaaacacacaagaaaaaaataatataattataaaagtatcattgtcttggaactcagttctatattaattctcatttttggtgtttatatatagaatactaagaggtactgcttctttgaaaagacacaacattttccttagaaaaaattatgaatagttatatatatttacgtaaagacacctctctttaattacatttttctttctttcctattatatatattataaataatataaaactttaatactatatattttatttgaaattactttataatatataatataaattatttatatgttatatattatatacaacaattattagtaagttaagattgaatcagaaaaaatattacgagtcaaatagttttttactttgttttataataaaaaagtaattaaaataaatttagccccaataaaaaaaattaaatctactctttaggtgaaatttttaattaattagtccctgaggtaagctttcggctgctaagctatgaaattgtcattatgtataacttttatgcaagtgtccctcacctctcggacacctccctccttcacaaaacagcgaggtgtacgctcacgtgtcaatgttgggttacgtgttaaggctccaacattccgatccaccggtcaatcccctctgtgtactctgtgtacataagctgtgccccatatacaaacaccaacggagctcaacaaagtatctgtacggtaccgcattatatttttattgacccaag